European Patent Specification EP 3 898 665 B1, published November 27, 2024. Title: CD-22-specific T cell receptors and adoptive T cell therapy for treatment of B cell malignancies. Applicant: Charité - Universitaetsmedizin Berlin Max-Delbrueck-Centrum fuer Molekulare Medizin. The sequence listing filed with the application follows.

SEQUENCE LISTING (27 sequences)

SEQ ID NO: 1 - protein, 9 aa, Homo sapiens
  FLS peptide: CD22 epitope
FLSNDTVQL

SEQ ID NO: 2 - protein, 6 aa, Homo sapiens
  alpha chain CDR1
VTNFRS

SEQ ID NO: 3 - protein, 7 aa, Homo sapiens
  alpha chain CDR2
LTSSGIE

SEQ ID NO: 4 - protein, 12 aa, Homo sapiens
  alpha chain CDR3
CAVDNQGGKLIF

SEQ ID NO: 5 - protein, 6 aa, Homo sapiens
  beta chain CDR1
DFQATT

SEQ ID NO: 6 - protein, 7 aa, Homo sapiens
  beta chain CDR2
SNEGSKA

SEQ ID NO: 7 - protein, 14 aa, Homo sapiens
  beta chain CDR3
CSARPSGVYNEQFF

SEQ ID NO: 8 - DNA, 411 bp, Artificial Sequence
  murine constant region of TCR alpha - codon-optimized
aacatccagaaccccgagcccgccgtgtaccagctgaaggaccccagaagccaggacagcaccctgtgcctgttcaccgacttcgacagccagatcaacgtgcccaagaccatggaaagcggcaccttcatcaccgacaagacagtgctggacatgaaggccatggacagcaagagcaacggcgccattgcctggtccaaccagaccagcttcacatgccaggacatcttcaaagagacaaacgccacctaccccagcagcgacgtgccctgcgacgccaccctgaccgagaagagcttcgagacagacatgaacctgaatttccagaacctgagcgtgatgggcctgcggatcctgctgctgaaggtggccggcttcaacctgctgatgaccctgcggctgtggagcagc

SEQ ID NO: 9 - DNA, 423 bp, Artificial Sequence
  minimally murinized constant region - TCR alpha
aacatccagaaccccgaccccgccgtgtatcagctgagagacagcaagagcagcgacaagtccgtgtgcctgttcaccgacttcgacagccagaccaatgtgtcccagtccaaggacagcgacgtgtacatcaccgacaagaccgtgctggacatgcgcagcatggacttcaagagcaactccgccgtggcctggtccaacaagagcgatttcgcctgcgccaacgccttcaacaacagcattatccccgaggacacattcttcccaagctcagacgttccctgcgacgtgaagctggtggaaaagagcttcgagacagacaccaacctgaacttccagaacctgagcgtgatcggcttccggatcctgctgctgaaggtggccggcttcaacctgctgatgaccctgagactgtggtccagc

SEQ ID NO: 10 - DNA, 423 bp, Artificial Sequence
  human constant region TCR alpha - codon-optimized
aacatccagaaccccgaccccgccgtgtatcagctgagagacagcaagagcagcgacaagtccgtgtgcctgttcaccgacttcgacagccagaccaatgtgtcccagtccaaggacagcgacgtgtacatcaccgacaagaccgtgctggacatgcgcagcatggacttcaagagcaactccgccgtggcctggtccaacaagagcgatttcgcctgcgccaacgccttcaacaacagcattatccccgaggacacattcttcccaagccccgagagcagctgcgacgtgaagctggtggaaaagagcttcgagacagacaccaacctgaacttccagaacctgagcgtgatcggcttccggatcctgctgctgaaggtggccggcttcaacctgctgatgaccctgagactgtggtccagc

SEQ ID NO: 11 - DNA, 519 bp, Artificial Sequence
  murine constant region TCR beta - codon optimized
gaagatctgaggaacgtgaccccacccaaggtgtccctgttcgagcccagcaaggccgagatcgccaacaagcagaaagccaccctggtctgcctggccaggggcttcttccccgaccacgtggagctgtcttggtgggtgaacggcaaagaggtgcacagcggagtcagtaccgacccccaggcctacaaagagagcaactacagctactgcctgagcagcaggctgagagtgagcgccaccttctggcacaacccccggaaccacttccggtgccaggtgcagttccacggcctgagcgaagaggacaagtggcctgagggcagccccaagcccgtgacccagaacatcagcgccgaggcctggggcagagccgactgcggcatcaccagcgccagctaccaccagggcgtgctgtccgccaccatcctgtacgagatcctgctgggcaaggccaccctgtacgccgtgctggtgtccggcctggtgctgatggccatggtgaagaagaagaacagc

SEQ ID NO: 12 - DNA, 537 bp, Artificial Sequence
  minimally murinized constant region TCR beta codon-optimized
gaggatctgaagaacgtgttccccccagaggtggccgtgttcgagccttctaaagccgagatcgcacacacccagaaagccaccctcgtgtgtctggccaccggcttctaccccgaccatgtggaactgtcttggtgggtcaacggcaaagaggtgcacagcggagtgtccaccgacccccagcctctgaaagaacagcccgccctgaacgacagccggtactgcctgagcagcagactgagagtgtccgccaccttctggcagaacccccggaaccacttcagatgccaggtgcagttctacggcctgagcgagaacgacgagtggacccaggacagagccaagcccgtgacccagatcgtgtctgccgaagcctggggcagagccgattgcggcatcaccagcgcaagctaccatcagggcgtgctgagcgccacaatcctgtacgagattctgctgggcaaggccacactgtacgccgtgctggtgtctgccctggtgctgatggccatggtcaagcggaaggacagcagaggc

SEQ ID NO: 13 - DNA, 537 bp, Artificial Sequence
  human constant region TCR beta - codon-optimized
gaggatctgaagaacgtgttccccccagaggtggccgtgttcgagccttctgaggccgagatcagccacacccagaaagccaccctcgtgtgtctggccaccggcttctaccccgaccatgtggaactgtcttggtgggtcaacggcaaagaggtgcacagcggagtgtccaccgacccccagcctctgaaagaacagcccgccctgaacgacagccggtactgcctgagcagcagactgagagtgtccgccaccttctggcagaacccccggaaccacttcagatgccaggtgcagttctacggcctgagcgagaacgacgagtggacccaggacagagccaagcccgtgacccagatcgtgtctgccgaagcctggggcagagccgattgcggctttaccagcgagagctaccagcagggcgtgctgagcgccacaatcctgtacgagattctgctgggcaaggccacactgtacgccgtgctggtgtctgccctggtgctgatggccatggtcaagcggaaggacagcagaggc

SEQ ID NO: 14 - DNA, 390 bp, Homo sapiens
  aCD22 TCR alpha chain variable region TRAV36/DV7*04-TRAJ23*01 incl. leader
atgaagtgtccacaggctttactagctatcttttggcttctactgagctgggtgagcagtgaagacaaggtggtacaaagccctctatctctggttgtccacgagggagacactgtaactctcaattgcagttatgaagtgactaactttcgaagcctactatggtacaagcaggaaaagaaagctcccacatttctatttatgctaacttcaagtggaattgaaaagaagtcaggaagactaagtagcatattagataagaaagaacttttcagcatcctgaacatcacagccacccagaccggagactcggccgtctacctctgtgctgtggataaccagggaggaaagcttatcttcggacagggaacggagttatctgtgaaaccc

SEQ ID NO: 15 - DNA, 390 bp, Artificial Sequence
  aCD22 TCR alpha chain variable region TRAV36/DV7*04-TRAJ23*01 - codon-optimized
atgaagtgcccacaggccctgctggccatcttttggctgctgctgagctgggtgtccagcgaggacaaggtggtgcagagccctctgagcctggtggtgcacgagggcgataccgtgaccctgaattgcagctacgaagtgaccaacttccggtccctgctgtggtacaagcaggaaaagaaggcccccaccttcctgttcatgctgaccagcagcggcatcgagaagaagtccggcagactgtcctccatcctggacaagaaagagctgttcagcatcctgaatatcaccgccacccagaccggcgacagcgccgtgtatctgtgcgccgtggataaccagggcggcaagctgatctttggccagggcacagagctgagcgtgaagccc

SEQ ID NO: 16 - protein, 130 aa, Artificial Sequence
  SIGNAL 1..20: leader
  aDC22 TCR alpha chain variable region TRAV36/DV7*04-TRAJ23*01 incl. leader
MKCPQALLAIFWLLLSWVSSEDKVVQSPLSLVVHEGDTVTLNCSYEVTNFRSLLWYKQEKKAPTFLFMLTSSGIEKKSGRLSSILDKKELFSILNITATQTGDSAVYLCAVDNQGGKLIFGQGTELSVKP

SEQ ID NO: 17 - DNA, 423 bp, Homo sapiens
  aCD22 TCR beta chain variable sequence TRBV20-1-TRBJ2-1*01-TRBD2*01 incl. leader
atgggggaaggtggtgtgaggccatcacggaagatgctgctgcttctgctgcttctggggccaggctccgggcttggtgctgtcgtctctcaacatccgagctgggttatctgtaagagtggaacctctgtgaagatcgagtgccgttccctggactttcaggccacaactatgttttggtatcgtcagttcccgaaacagagtctcatgctgatggcaacttccaatgagggctccaaggccacatacgagcaaggcgtcgagaaggacaagtttctcatcaaccatgcaagcctgaccttgtccactctgacagtgaccagtgcccatcctgaagacagcagcttctacatctgcagtgctaggcctagcggggtctacaatgagcagttcttcgggccagggacacggctcaccgtgcta

SEQ ID NO: 18 - DNA, 423 bp, Artificial Sequence
  aCD22 TCR beta chain variable region TRBV20-1-TRBJ2-1*01-TRBD2*01 incl. leader - codon optimized
atgggagaaggcggagtgcggcctagccggaagatgcttctccttctgctgctgctgggccctggctctggactgggagctgtggtgtctcagcacccctcctgggtcatctgcaagagcggcaccagcgtgaagatcgagtgcagaagcctggacttccaggccaccaccatgttctggtacagacagttccccaagcagagcctgatgctgatggccacctccaacgagggcagcaaggccacatatgagcagggcgtggaaaaggacaagttcctgatcaaccacgccagcctgaccctgagcaccctgacagtgacaagcgcccaccccgaggacagcagcttctacatctgcagcgccagacccagcggcgtgtacaacgagcagttcttcggccctggcacccggctgaccgtgctg

SEQ ID NO: 19 - protein, 141 aa, Artificial Sequence
  SIGNAL 1..25: Leader sequence aa12-25, TCR sequence starts at aa 26
  aCD22 TCR beta chain variable region TRBV20-1-TRBJ2-1*01-TRBD2*01 incl. leader
MGEGGVRPSRKMLLLLLLLGPGSGLGAVVSQHPSWVICKSGTSVKIECRSLDFQATTMFWYRQFPKQSLMLMATSNEGSKATYEQGVEKDKFLINHASLTLSTLTVTSAHPEDSSFYICSARPSGVYNEQFFGPGTRLTVL

SEQ ID NO: 20 - protein, 6 aa, Homo sapiens
  beta chain CDR1
DFQATT

SEQ ID NO: 21 - protein, 7 aa, Homo sapiens
  beta chain CDR2
SNEGSKA

SEQ ID NO: 22 - protein, 14 aa, Homo sapiens
  3225 TCR beta chain CDR3
CSAREAGVYNEQFF

SEQ ID NO: 23 - DNA, 390 bp, Homo sapiens
  3225 TCR beta chain variable region TRBV20-1*01-TRBJ2-1*01-TRBD2*02 F incl. leader
  sig_peptide 1..42: /function="leader peptide"
atgctgctgcttctgctgcttctggggccaggctccgggcttggtgctgtcgtctctcaacatccgagctgggttatctgtaagagtggaacctctgtgaagatcgagtgccgttccctggactttcaggccacaactatgttttggtatcgtcagttcccgaaacagagtctcatgctgatggcaacttccaatgagggctccaaggccacatacgagcaaggcgtcgagaaggacaagtttctcatcaaccatgcaagcctgaccttgtccactctgacagtgaccagtgcccatcctgaagacagcagcttctacatctgcagtgctagagaagcgggagtctacaatgagcagttcttcgggccagggacacggctcaccgtgcta

SEQ ID NO: 24 - DNA, 390 bp, Artificial Sequence
  3225 TCR beta chain variable region codon-optimized TRBV20-1*01-TRBJ2-1*01-TRBD2*02 F
  sig_peptide 1..42: /function="leader peptide"
atgcttctccttctgctgctgctgggccctggctctggactgggagctgtggtgtctcagcacccctcctgggtcatctgcaagagcggcaccagcgtgaagatcgagtgcagaagcctggacttccaggccaccaccatgttctggtacagacagttccccaagcagagcctgatgctgatggccacctccaacgagggcagcaaggccacatatgagcagggcgtggaaaaggacaagttcctgatcaaccacgccagcctgaccctgagcaccctgacagtgacaagcgcccaccccgaggacagcagcttctacatctgcagcgccagagaagcgggcgtgtacaacgagcagttcttcggccctggcacccggctgaccgtgctg

SEQ ID NO: 25 - protein, 130 aa, Homo sapiens
  SIGNAL 1..14: leader peptide
  3225 TCR beta chain variable region TRBV20-1*01-TRBJ2-1*01-TRBD2*02 F incl. leader
MLLLLLLLGPGSGLGAVVSQHPSWVICKSGTSVKIECRSLDFQATTMFWYRQFPKQSLMLMATSNEGSKATYEQGVEKDKFLINHASLTLSTLTVTSAHPEDSSFYICSAREAGVYNEQFFGPGTRLTVL

SEQ ID NO: 26 - DNA, 42 bp, Homo sapiens
  3225 beta chain construct CDR3 nt
tgcagtgctagagaagcgggagtctacaatgagcagttcttc

SEQ ID NO: 27 - DNA, 42 bp, Artificial Sequence
  3225 beta chain construct CDR3 nt codon optimized
tgcagcgccagagaagcgggcgtgtacaacgagcagttcttc